European Patent Application EP 4 703 471 A1, published March 4, 2026. Title: Method for Controlling Transription and/or Replication of vRNA with RdRp of Influenza Virus, and Use thereof. Applicant: SHINSHU UNIVERSITY. The sequence listing filed with the application follows.

SEQUENCE LISTING (2 sequences)

SEQ ID NO: 1 - protein, 19 aa, Porcine teschovirus
ATNFSLLKQAGDVEENPGP

SEQ ID NO: 2 - protein, 28 aa, synthetic construct
WSHPQFEKGGGSGGGSGGSAWSHPQFEK